European Patent Application EP 4 458 954 A1, published November 6, 2024. Title: Culture method and menufacturing method of neural crest cells. Applicant: 住友ファーマ株式会社. The sequence listing filed with the application follows.

SEQUENCE LISTING (10 sequences)

SEQ ID NO: 1 - DNA, 20 bp, synthetic construct
  source 1..20: mol_type = other DNA
ccgttggattacacggtcca

SEQ ID NO: 2 - DNA, 20 bp, synthetic construct
  source 1..20: mol_type = other DNA
gacagggatgaggttgtcgg

SEQ ID NO: 3 - DNA, 20 bp, synthetic construct
  source 1..20: mol_type = other DNA
agggcctcggtgagatagtt

SEQ ID NO: 4 - DNA, 20 bp, synthetic construct
  source 1..20: mol_type = other DNA
aagagttcaccgacctgctg

SEQ ID NO: 5 - DNA, 20 bp, synthetic construct
  source 1..20: mol_type = other DNA
ttttaaaagtgcgccccacg

SEQ ID NO: 6 - DNA, 20 bp, synthetic construct
  source 1..20: mol_type = other DNA
tctcggtctggaggatggag

SEQ ID NO: 7 - DNA, 22 bp, synthetic construct
  source 1..22: mol_type = other DNA
gagctggaccgcacaccttggg

SEQ ID NO: 8 - DNA, 22 bp, synthetic construct
  source 1..22: mol_type = other DNA
aacgcccacctcctcggacctc

SEQ ID NO: 9 - DNA, 17 bp, synthetic construct
  source 1..17: mol_type = other DNA
gagcagacgcacatctc

SEQ ID NO: 10 - DNA, 16 bp, synthetic construct
  source 1..16: mol_type = other DNA
cctgggattgccccga